European Patent Application EP 4 538 374 A1, published April 16, 2025. Title: METHOD FOR PRECISELY PREPARING CIRCULAR RNA WITH ANABAENA INTRON SELF-CLEAVING RIBOZYME. Applicant: Guangzhou Geneseed Biotech Co.,Ltd. The sequence listing filed with the application follows.

SEQUENCE LISTING (9 sequences)

SEQ ID NO: 1 - RNA, 313 nt, synthetic construct
  source 1..313: mol_type = other RNA; note = Anabaena intronic self-cleaving ribozyme sequence
tgcggaatggtagacgctacggacttaaataattgagccttaaagaagaaattctttaagtggatgctctcaaactcagggaaacctaaatctagttatagacaaggcaatcctgagccaagccgaagtagtaattagtaagttaacaatagatgacttacaactaatcggaaggtgcagagactcgacgggagctaccctaacgtcaagacgagggtaaagagagagtccaattctcaaagccaataggcagtagcgaaagctgcaagagaatgaaaatccgttgaccttaaacggtcgtgtgggttcaagt

SEQ ID NO: 2 - RNA, 246 nt, synthetic construct
  source 1..246: mol_type = other RNA; note = artificial sequence
attaatcatcatcctagccctaagtctggcctatgagtgactacaactcaacggctacatagaaaaatccaccccttacgagtgcggcttcgaccctatatcccccgcccgcgtccctttctccataaaattcttcttagtagctattaccttcttattatttgatctagaaattgccctccttttacccctaccatgagccctacaaacaactaacctgccactaatagttatgtcatccctctt

SEQ ID NO: 3 - RNA, 493 nt, synthetic construct
  source 1..493: mol_type = other RNA
aacaatagatgacttacaactaatcggaaggtgcagagactcgacgggagctaccctaacgtcaagacgagggtaaagagagagtccaattctcaaagccaataggcagtagcgaaagctgcaagagaatgattaatcatcatcctagccctaagtctggcctatgagtgactacaactcaacggctacatagaaaaatccaccccttacgagtgcggcttcgaccctatatcccccgcccgcgtccctttctccataaaattcttcttagtagctattaccttcttattatttgatctagaaattgccctccttttacccctaccatgagccctacaaacaactaacctgccactaatagttatgtcatccctcttaaataattgagccttaaagaagaaattctttaagtggatgctctcaaactcagggaaacctaaatctagttatagacaaggcaatcctgagccaagccgaagtagtaattagtaag

SEQ ID NO: 4 - DNA, 18 bp, synthetic construct
  source 1..18: mol_type = other DNA
cacggacagaccgccggc

SEQ ID NO: 5 - DNA, 18 bp, synthetic construct
  source 1..18: mol_type = other DNA
gccggcggtctgtccgtg

SEQ ID NO: 6 - DNA, 20 bp, synthetic construct
  source 1..20: mol_type = other DNA
taatacgactcactataggg

SEQ ID NO: 7 - DNA, 561 bp, synthetic construct
  source 1..561: mol_type = other DNA
ggatcctaatacgactcactatagggcacggacagaccgccggcaacaatagatgacttacaactaatcggaaggtgcagagactcgacgggagctaccctaacgtcaagacgagggtaaagagagagtccaattctcaaagccaataggcagtagcgaaagctgcaagagaatgattaatcatcatcctagccctaagtctggcctatgagtgactacaactcaacggctacatagaaaaatccaccccttacgagtgcggcttcgaccctatatcccccgcccgcgtccctttctccataaaattcttcttagtagctattaccttcttattatttgatctagaaattgccctccttttacccctaccatgagccctacaaacaactaacctgccactaatagttatgtcatccctcttaaataattgagccttaaagaagaaattctttaagtggatgctctcaaactcagggaaacctaaatctagttatagacaaggcaatcctgagccaagccgaagtagtaattagtaaggccggcggtctgtccgtggaattc

SEQ ID NO: 8 - DNA, 20 bp, synthetic construct
  source 1..20: mol_type = other DNA
ctccttttacccctaccatg

SEQ ID NO: 9 - DNA, 18 bp, synthetic construct
  source 1..18: mol_type = other DNA
gatatagggtcgaagccg